European Patent Application EP 4 745 232 A2, published May 20, 2026. Title: LEISTUNGSVERBESSERTE PROTEASE-VARIANTEN. Applicant: Henkel AG & Co. KGaA. Application EP. The sequence listing filed with the application follows.

SEQUENCE LISTING (1 sequence)

SEQ ID NO: 1 - protein, 269 aa, Bacillus gibsonii
QQTVPWGITRVQAPTVHNRGITGSGVKVAILDTGIAQHSDLTIRGGASFVPGESTTADLNGHGTHVAGTVAALNNSIGVIGVAPSADLYAVKVLGANGRGSVSGIAQGLEWAATNNMHIANMSLGSDAPSTTLERAVNYATSRGVLVIAATGNNGTGSIGYPARYANAMAVGATDQNNRRASFSQYGTGIDIVAPGVGIQSTYLNNSYASMPGTSMATPHVAGVAALVKQKNPSWNATQIRNHLKNTATNLGNSSQFGSGLVNADAATR